European Patent Application EP 4 559 937 A1, published May 28, 2025. Title: CD7 TARGETING MOIETIES FOR THE TRATMENT OF CD7 POSITIVE CANCER. Applicant: Universitat de Barcelona. The sequence listing filed with the application follows.

SEQUENCE LISTING (77 sequences)

SEQ ID NO: 1 - protein, 107 aa, synthetic construct
DILLTQSPAILSVSPGERVSFSCRASQSIGTSIHWYQQRTNDSPRLLIKYASESISGIPSRFSGSGSGTDFTLNINSVESEDIADYYCQQSISWPLTFGPGTKLELK

SEQ ID NO: 2 - protein, 119 aa, synthetic construct
DVQLQESGPGLVKPSQSLSLTCTVTGYSITSDYAWNWIRQFPGNKLEWLGYISYSGSTSYNPSLKSRISITRDTSKNQFFLQLNSVTTEDTATYYCAKSQLGRWAMDYWGQGTSVTVSS

SEQ ID NO: 3 - protein, 267 aa, synthetic construct
MALPVTGLLLSLGLLLHAARPDILLTQSPAILSVSPGERVSFSCRASQSIGTSIHWYQQRTNDSPRLLIKYASESISGIPSRFSGSGSGTDFTLNINSVESEDIADYYCQQSISWPLTFGPGTKLELKGGGGSGGGGSGGGGSGGGGSDVQLQESGPGLVKPSQSLSLTCTVTGYSITSDYAWNWIRQFPGNKLEWLGYISYSGSTSYNPSLKSRISITRDTSKNQFFLQLNSVTTEDTATYYCAKSQLGRWAMDYWGQGTSVTVSS

SEQ ID NO: 4 - protein, 11 aa, synthetic construct
RASQSIGTSIH

SEQ ID NO: 5 - protein, 7 aa, synthetic construct
YASESIS

SEQ ID NO: 6 - protein, 9 aa, synthetic construct
QQSISWPLT

SEQ ID NO: 7 - protein, 6 aa, synthetic construct
SDYAWN

SEQ ID NO: 8 - protein, 16 aa, synthetic construct
YISYSGSTSYNPSLKS

SEQ ID NO: 9 - protein, 10 aa, synthetic construct
SQLGRWAMDY

SEQ ID NO: 10 - protein, 20 aa, synthetic construct
GGGGSGGGGSGGGGSGGGGS

SEQ ID NO: 11 - protein, 267 aa, synthetic construct
MALPVTGLLLSLGLLLHAARPDILLTQSPAILSVSPGERVSFSCRASQNIGTSIHWFQQRSNGSPSLLIKYASESMSGIPSRFSGSGSGTDFTLSINSVEPEDIADYYCQQSNRWPYTFGGGTKLEIKGGGGSGGGGSGGGGSGGGGSQLVQSGPEVKKPGETVKISCKASGYSFTHYGVNWVKQAPGKGLKWMGWINTNTGKPTYAEDFKGRFAFSLETSARTAYLQINNLKNEDTATYFCARWSTTVVAPYFDVWGAGTTVTVSS

SEQ ID NO: 12 - protein, 491 aa, synthetic construct
MALPVTGLLLSLGLLLHAARPDILLTQSPAILSVSPGERVSFSCRASQNIGTSIHWFQQRSNGSPSLLIKYASESMSGIPSRFSGSGSGTDFTLSINSVEPEDIADYYCQQSNRWPYTFGGGTKLEIKGGGGSGGGGSGGGGSGGGGSQLVQSGPEVKKPGETVKISCKASGYSFTHYGVNWVKQAPGKGLKWMGWINTNTGKPTYAEDFKGRFAFSLETSARTAYLQINNLKNEDTATYFCARWSTTVVAPYFDVWGAGTTVTVSSTTTPAPRPPTPAPTIASQPLSLRPEACRPAAGGAVHTRGLDFACDIYIWAPLAGTCGVLLLSLVITLYCKRGRKKLLYIFKQPFMRPVQTTQEEDGCSCRFPEEEEGGCELRVKFSRSADAPAYQQGQNQLYNELNLGRREEYDVLDKRRGRDPEMGGKPQRRKNPQEGLYNELQKDKMAEAYSEIGMKGERRRGKGHDGLYQGLSTATKDTYDALHMQALPPR

SEQ ID NO: 13 - protein, 491 aa, synthetic construct
MALPVTGLLLSLGLLLHAARPDILLTQSPAILSVSPGERVSFSCRASQSIGTSIHWYQQRTNDSPRLLIKYASESISGIPSRFSGSGSGTDFTLNINSVESEDIADYYCQQSISWPLTFGPGTKLELKGGGGSGGGGSGGGGSGGGGSDVQLQESGPGLVKPSQSLSLTCTVTGYSITSDYAWNWIRQFPGNKLEWLGYISYSGSTSYNPSLKSRISITRDTSKNQFFLQLNSVTTEDTATYYCAKSQLGRWAMDYWGQGTSVTVSSTTTPAPRPPTPAPTIASQPLSLRPEACRPAAGGAVHTRGLDFACDIYIWAPLAGTCGVLLLSLVITLYCKRGRKKLLYIFKQPFMRPVQTTQEEDGCSCRFPEEEEGGCELRVKFSRSADAPAYQQGQNQLYNELNLGRREEYDVLDKRRGRDPEMGGKPQRRKNPQEGLYNELQKDKMAEAYSEIGMKGERRRGKGHDGLYQGLSTATKDTYDALHMQALPPR

SEQ ID NO: 14 - protein, 11 aa, synthetic construct
RASQNIGTSIH

SEQ ID NO: 15 - protein, 7 aa, synthetic construct
YASESMS

SEQ ID NO: 16 - protein, 9 aa, synthetic construct
QQSNRWPYT

SEQ ID NO: 17 - protein, 5 aa, synthetic construct
HYGVN

SEQ ID NO: 18 - protein, 17 aa, synthetic construct
WINTNTGKPTYAEDFKG

SEQ ID NO: 19 - protein, 12 aa, synthetic construct
WSTTVVAPYFDV

SEQ ID NO: 20 - protein, 107 aa, synthetic construct
DILLTQSPAILSVSPGERVSFSCRASQNIGTSIHWFQQRSNGSPSLLIKYASESMSGIPSRFSGSGSGTDFTLSINSVEPEDIADYYCQQSNRWPYTFGGGTKLEIK

SEQ ID NO: 21 - protein, 119 aa, synthetic construct
QLVQSGPEVKKPGETVKISCKASGYSFTHYGVNWVKQAPGKGLKWMGWINTNTGKPTYAEDFKGRFAFSLETSARTAYLQINNLKNEDTATYFCARWSTTVVAPYFDVWGAGTTVTVSS

SEQ ID NO: 22 - protein, 24 aa, synthetic construct
IYIWAPLAGTCGVLLLSLVITLYC

SEQ ID NO: 23 - protein, 45 aa, synthetic construct
TTTPAPRPPTPAPTIASQPLSLRPEACRPAAGGAVHTRGLDFACD

SEQ ID NO: 24 - protein, 69 aa, synthetic construct
TTTPAPRPPTPAPTIASQPLSLRPEACRPAAGGAVHTRGLDFACDIYIWAPLAGTCGVLLLSLVITLYC

SEQ ID NO: 25 - protein, 113 aa, synthetic construct
RVKFSRSADAPAYQQGQNQLYNELNLGRREEYDVLDKRRGRDPEMGGKPQRRKNPQEGLYNELQKDKMAEAYSEIGMKGERRRGKGHDGLYQGLSTATKDTYDALHMQALPPR

SEQ ID NO: 26 - protein, 42 aa, synthetic construct
KRGRKKLLYIFKQPFMRPVQTTQEEDGCSCRFPEEEEGGCEL

SEQ ID NO: 27 - protein, 21 aa, synthetic construct
MALPVTGLLLSLGLLLHAARP

SEQ ID NO: 28 - protein, 1476 aa, synthetic construct
ATGGCTCTGCCTGTAACCGGACTCTTACTCTCTTTGGGGCTACTCCTTCACGCAGCCAGGCCTGACATTCTGCTGACTCAGTCACCAGCCATCCTCTCAGTGTCACCTGGCGAGCGTGTTTCATTCAGCTGTAGGGCTTCGCAAAATATCGGGACCAGCATCCACTGGTTCCAGCAGAGATCTAACGGCTCGCCAAGCTTACTCATCAAATATGCGAGTGAGTCCATGTCCGGCATCCCTTCACGCTTTTCCGGCTCTGGTTCTGGAACTGATTTTACCCTTAGCATAAATAGTGTGGAGCCTGAAGATATAGCCGACTACTACTGCCAACAATCCAACCGGTGGCCCTACACATTTGGCGGTGGCACCAAACTTGAGATTAAGGGTGGGGGGGGTAGCGGAGGAGGCGGATCAGGAGGGGGCGGCAGTGGAGGCGGGGGCTCCCAGCTAGTGCAGTCTGGACCCGAAGTGAAAAAGCCTGGAGAGACAGTTAAGATTTCCTGCAAAGCAAGTGGATATAGCTTCACACACTACGGTGTAAATTGGGTGAAGCAGGCACCAGGCAAAGGGCTTAAGTGGATGGGGTGGATCAACACAAATACGGGCAAGCCCACTTATGCCGAAGACTTTAAGGGGAGATTCGCCTTCTCTCTGGAAACGAGTGCACGAACAGCTTACCTCCAGATTAACAATCTGAAAAACGAGGATACTGCTACATATTTCTGTGCTAGGTGGTCAACCACCGTCGTGGCCCCCTACTTTGACGTCTGGGGTGCGGGGACTACCGTAACCGTCTCCTCCACAACTACGCCGGCGCCGAGACCACCTACACCTGCACCAACTATTGCCTCTCAGCCACTGAGTCTGCGCCCCGAGGCATGTCGACCTGCCGCTGGCGGGGCTGTGCACACCAGGGGCCTAGACTTCGCCTGCGATATCTATATTTGGGCTCCACTGGCAGGAACCTGTGGCGTGCTGCTGCTGTCTCTGGTCATCACACTGTACTGCAAAAGAGGCAGGAAGAAACTGCTGTATATTTTCAAGCAGCCCTTTATGAGACCTGTGCAGACAACTCAGGAGGAAGACGGGTGCAGCTGTAGGTTCCCTGAGGAAGAGGAAGGAGGCTGTGAGCTGCGCGTGAAATTTTCTCGGAGTGCAGATGCCCCAGCTTACCAGCAGGGCCAGAACCAGCTGTATAACGAGCTGAATCTGGGGCGGAGAGAGGAATACGACGTGCTGGATAAGAGGCGCGGGCGAGATCCAGAAATGGGAGGAAAACCCCAGCGACGGAAGAACCCTCAGGAGGGACTGTACAATGAACTGCAGAAGGACAAAATGGCAGAGGCCTATTCCGAAATCGGGATGAAAGGAGAAAGAAGGCGCGGCAAGGGGCATGATGGCCTGTATCAGGGACTGTCAACCGCAACAAAAGATACTTATGATGCTCTGCACATGCAGGCTCTGCCCCCGCGGTAA

SEQ ID NO: 29 - protein, 20 aa, synthetic construct
SREGRGSLLTCGDVEENPGP

SEQ ID NO: 30 - protein, 6 aa, synthetic construct
AEKDEL

SEQ ID NO: 31 - protein, 293 aa, synthetic construct
MALPVTGLLLSLGLLLHAARPDILLTQSPAILSVSPGERVSFSCRASQSIGTSIHWYQQRTNDSPRLLIKYASESISGIPSRFSGSGSGTDFTLNINSVESEDIADYYCQQSISWPLTFGPGTKLELKGGGGSGGGGSGGGGSGGGGSDVQLQESGPGLVKPSQSLSLTCTVTGYSITSDYAWNWIRQFPGNKLEWLGYISYSGSTSYNPSLKSRISITRDTSKNQFFLQLNSVTTEDTATYYCAKSQLGRWAMDYWGQGTSVTVSSGGGGSGGGGSGGGGSGGGGSAEKDEL

SEQ ID NO: 32 - protein, 293 aa, synthetic construct
MALPVTGLLLSLGLLLHAARPDILLTQSPAILSVSPGERVSFSCRASQNIGTSIHWFQQRSNGSPSLLIKYASESMSGIPSRFSGSGSGTDFTLSINSVEPEDIADYYCQQSNRWPYTFGGGTKLEIKGGGGSGGGGSGGGGSGGGGSQLVQSGPEVKKPGETVKISCKASGYSFTHYGVNWVKQAPGKGLKWMGWINTNTGKPTYAEDFKGRFAFSLETSARTAYLQINNLKNEDTATYFCARWSTTVVAPYFDVWGAGTTVTVSSGGGGSGGGGSGGGGSGGGGSAEKDEL

SEQ ID NO: 33 - protein, 882 aa, synthetic construct
ATGGCTCTGCCTGTAACCGGACTCTTACTCTCTTTGGGGCTACTCCTTCACGCAGCCAGGCCTGACATTCTGCTTACACAGAGTCCCGCCATCCTGAGCGTCTCTCCAGGCGAGCGGGTCTCCTTCAGTTGTCGCGCTAGTCAGAGCATTGGAACCTCCATCCATTGGTATCAGCAGAGAACGAATGATAGCCCCCGGCTGCTGATAAAGTATGCATCCGAGTCCATATCAGGCATCCCTTCTAGGTTTTCAGGAAGCGGATCTGGCACTGACTTTACGTTGAACATCAACAGCGTGGAATCCGAGGACATCGCTGATTATTATTGCCAACAGTCTATCTCCTGGCCGCTTACATTCGGCCCAGGAACAAAGTTAGAGCTGAAGGGTGGGGGGGGTAGCGGAGGAGGCGGATCAGGAGGGGGCGGCAGTGGAGGCGGGGGCTCCGATGTGCAGCTGCAAGAAAGTGGCCCAGGTCTTGTGAAGCCTAGTCAGAGCCTGAGCCTAACCTGTACAGTGACCGGTTACAGCATTACTTCGGATTACGCATGGAACTGGATTCGTCAATTCCCCGGTAACAAACTGGAGTGGCTCGGATACATCAGCTATTCCGGGTCCACATCCTACAATCCCTCTTTGAAATCCAGAATATCTATTACACGAGACACCAGCAAGAATCAATTCTTTCTGCAGTTGAATTCAGTGACCACCGAAGACACCGCCACTTACTACTGCGCGAAATCACAGCTGGGGAGATGGGCCATGGATTACTGGGGGCAGGGGACTAGCGTTACTGTTTCTTCAGGCGGTGGCGGATCAGGTGGGGGCGGGTCTGGGGGCGGTGGCTCGGGCGGCGGGGGAAGTGCCGAGAAAGACGAACTCTAA

SEQ ID NO: 34 - protein, 882 aa, synthetic construct
ATGGCTCTGCCTGTAACCGGACTCTTACTCTCTTTGGGGCTACTCCTTCACGCAGCCAGGCCTGACATTCTGCTGACTCAGTCACCAGCCATCCTCTCAGTGTCACCTGGCGAGCGTGTTTCATTCAGCTGTAGGGCTTCGCAAAATATCGGGACCAGCATCCACTGGTTCCAGCAGAGATCTAACGGCTCGCCAAGCTTACTCATCAAATATGCGAGTGAGTCCATGTCCGGCATCCCTTCACGCTTTTCCGGCTCTGGTTCTGGAACTGATTTTACCCTTAGCATAAATAGTGTGGAGCCTGAAGATATAGCCGACTACTACTGCCAACAATCCAACCGGTGGCCCTACACATTTGGCGGTGGCACCAAACTTGAGATTAAGGGTGGGGGGGGTAGCGGAGGAGGCGGATCAGGAGGGGGCGGCAGTGGAGGCGGGGGCTCCCAGCTAGTGCAGTCTGGACCCGAAGTGAAAAAGCCTGGAGAGACAGTTAAGATTTCCTGCAAAGCAAGTGGATATAGCTTCACACACTACGGTGTAAATTGGGTGAAGCAGGCACCAGGCAAAGGGCTTAAGTGGATGGGGTGGATCAACACAAATACGGGCAAGCCCACTTATGCCGAAGACTTTAAGGGGAGATTCGCCTTCTCTCTGGAAACGAGTGCACGAACAGCTTACCTCCAGATTAACAATCTGAAAAACGAGGATACTGCTACATATTTCTGTGCTAGGTGGTCAACCACCGTCGTGGCCCCCTACTTTGACGTCTGGGGTGCGGGGACTACCGTAACCGTCTCCTCCGGCGGTGGCGGATCAGGTGGGGGCGGGTCTGGGGGCGGTGGCTCGGGCGGCGGGGGAAGTGCCGAGAAAGACGAACTCTAA

SEQ ID NO: 35 - protein, 19 aa, synthetic construct
ATNFSLLKQAGDVEENPGP

SEQ ID NO: 36 - protein, 20 aa, synthetic construct
QCTNYALLKLAGDVESNPGP

SEQ ID NO: 37 - protein, 22 aa, synthetic construct
VKQTLNFDLLKLAGDVESNPGP

SEQ ID NO: 38 - protein, 321 aa, synthetic construct
GACATTCTGCTTACACAGAGTCCCGCCATCCTGAGCGTCTCTCCAGGCGAGCGGGTCTCCTTCAGTTGTCGCGCTAGTCAGAGCATTGGAACCTCCATCCATTGGTATCAGCAGAGAACGAATGATAGCCCCCGGCTGCTGATAAAGTATGCATCCGAGTCCATATCAGGCATCCCTTCTAGGTTTTCAGGAAGCGGATCTGGCACTGACTTTACGTTGAACATCAACAGCGTGGAATCCGAGGACATCGCTGATTATTATTGCCAACAGTCTATCTCCTGGCCGCTTACATTCGGCCCAGGAACAAAGTTAGAGCTGAAG

SEQ ID NO: 39 - protein, 357 aa, synthetic construct
GATGTGCAGCTGCAAGAAAGTGGCCCAGGTCTTGTGAAGCCTAGTCAGAGCCTGAGCCTAACCTGTACAGTGACCGGTTACAGCATTACTTCGGATTACGCATGGAACTGGATTCGTCAATTCCCCGGTAACAAACTGGAGTGGCTCGGATACATCAGCTATTCCGGGTCCACATCCTACAATCCCTCTTTGAAATCCAGAATATCTATTACACGAGACACCAGCAAGAATCAATTCTTTCTGCAGTTGAATTCAGTGACCACCGAAGACACCGCCACTTACTACTGCGCGAAATCACAGCTGGGGAGATGGGCCATGGATTACTGGGGGCAGGGGACTAGCGTTACTGTTTCTTCA

SEQ ID NO: 40 - protein, 321 aa, synthetic construct
GACATTCTGCTGACTCAGTCACCAGCCATCCTCTCAGTGTCACCTGGCGAGCGTGTTTCATTCAGCTGTAGGGCTTCGCAAAATATCGGGACCAGCATCCACTGGTTCCAGCAGAGATCTAACGGCTCGCCAAGCTTACTCATCAAATATGCGAGTGAGTCCATGTCCGGCATCCCTTCACGCTTTTCCGGCTCTGGTTCTGGAACTGATTTTACCCTTAGCATAAATAGTGTGGAGCCTGAAGATATAGCCGACTACTACTGCCAACAATCCAACCGGTGGCCCTACACATTTGGCGGTGGCACCAAACTTGAGATTAAG

SEQ ID NO: 41 - protein, 357 aa, synthetic construct
CAGCTAGTGCAGTCTGGACCCGAAGTGAAAAAGCCTGGAGAGACAGTTAAGATTTCCTGCAAAGCAAGTGGATATAGCTTCACACACTACGGTGTAAATTGGGTGAAGCAGGCACCAGGCAAAGGGCTTAAGTGGATGGGGTGGATCAACACAAATACGGGCAAGCCCACTTATGCCGAAGACTTTAAGGGGAGATTCGCCTTCTCTCTGGAAACGAGTGCACGAACAGCTTACCTCCAGATTAACAATCTGAAAAACGAGGATACTGCTACATATTTCTGTGCTAGGTGGTCAACCACCGTCGTGGCCCCCTACTTTGACGTCTGGGGTGCGGGGACTACCGTAACCGTCTCCTCC

SEQ ID NO: 42 - protein, 10 aa, synthetic construct
SARSSVSYMN

SEQ ID NO: 43 - protein, 7 aa, synthetic construct
GISNLAS

SEQ ID NO: 44 - protein, 9 aa, synthetic construct
QLRSSYSRT

SEQ ID NO: 45 - protein, 5 aa, synthetic construct
NYWLG

SEQ ID NO: 46 - protein, 17 aa, synthetic construct
DFYPGSIYTNYNENFQG

SEQ ID NO: 47 - protein, 12 aa, synthetic construct
EGDYYGSGHFDY

SEQ ID NO: 48 - protein, 106 aa, synthetic construct
EILLTQSPAIIAASPGEKVTITCSARSSVSYMNWYQQKSGSSPKIWIYGISNLASGVPARFSGSGSGTSFSFTINSMEAEDVAYYYCQLRSSYSRTFGGGTKLEIK

SEQ ID NO: 49 - protein, 318 aa, synthetic construct
GAGATTCTGTTAACTCAGTCACCCGCTATTATTGCCGCATCTCCAGGCGAAAAGGTGACAATCACCTGCTCAGCCCGCAGCTCCGTATCTTACATGAACTGGTATCAGCAGAAATCAGGTTCATCCCCTAAGATATGGATCTATGGAATATCTAACTTGGCTTCAGGCGTGCCTGCAAGGTTCTCTGGGTCCGGTAGTGGCACTTCCTTTAGTTTCACAATCAATTCCATGGAAGCCGAGGATGTCGCATACTATTACTGTCAACTCAGAAGTTCCTACTCCCGTACATTCGGCGGCGGCACAAAACTTGAGATCAAG

SEQ ID NO: 50 - protein, 121 aa, synthetic construct
QVQLQQSGAELVRPGTSVKISCKASGYTFTNYWLGWVKQRPGHGLEWIGDFYPGSIYTNYNENFQGKATLTADTSSSTAYMQLSSLTSEDSAVYFCAREGDYYGSGHFDYWGQGTTLTVSS

SEQ ID NO: 51 - protein, 363 aa, synthetic construct
CAGGTGCAGCTCCAGCAGTCCGGTGCCGAGCTGGTTCGGCCCGGCACATCCGTGAAGATCTCCTGCAAGGCTTCGGGCTATACTTTCACCAACTATTGGCTGGGATGGGTGAAACAAAGGCCCGGTCACGGGTTGGAGTGGATCGGGGATTTCTACCCTGGATCAATTTATACCAATTATAACGAGAATTTTCAAGGGAAAGCTACACTGACCGCCGACACTAGCAGCAGCACCGCCTACATGCAGCTCAGCTCTCTTACGAGCGAGGACTCGGCCGTCTACTTTTGTGCACGAGAAGGGGACTACTACGGCAGTGGTCATTTTGATTACTGGGGGCAGGGTACCACCCTCACGGTCAGCTCT

SEQ ID NO: 52 - protein, 268 aa, synthetic construct
MALPVTGLLLSLGLLLHAARPEILLTQSPAIIAASPGEKVTITCSARSSVSYMNWYQQKSGSSPKIWIYGISNLASGVPARFSGSGSGTSFSFTINSMEAEDVAYYYCQLRSSYSRTFGGGTKLEIKGGGGSGGGGSGGGGSGGGGSQVQLQQSGAELVRPGTSVKISCKASGYTFTNYWLGWVKQRPGHGLEWIGDFYPGSIYTNYNENFQGKATLTADTSSSTAYMQLSSLTSEDSAVYFCAREGDYYGSGHFDYWGQGTTLTVSS

SEQ ID NO: 53 - protein, 1476 aa, synthetic construct
ATGGCTCTGCCTGTAACCGGACTCTTACTCTCTTTGGGGCTACTCCTTCACGCAGCCAGGCCTGACATTCTGCTTACACAGAGTCCCGCCATCCTGAGCGTCTCTCCAGGCGAGCGGGTCTCCTTCAGTTGTCGCGCTAGTCAGAGCATTGGAACCTCCATCCATTGGTATCAGCAGAGAACGAATGATAGCCCCCGGCTGCTGATAAAGTATGCATCCGAGTCCATATCAGGCATCCCTTCTAGGTTTTCAGGAAGCGGATCTGGCACTGACTTTACGTTGAACATCAACAGCGTGGAATCCGAGGACATCGCTGATTATTATTGCCAACAGTCTATCTCCTGGCCGCTTACATTCGGCCCAGGAACAAAGTTAGAGCTGAAGGGTGGGGGGGGTAGCGGAGGAGGCGGATCAGGAGGGGGCGGCAGTGGAGGCGGGGGCTCCGATGTGCAGCTGCAAGAAAGTGGCCCAGGTCTTGTGAAGCCTAGTCAGAGCCTGAGCCTAACCTGTACAGTGACCGGTTACAGCATTACTTCGGATTACGCATGGAACTGGATTCGTCAATTCCCCGGTAACAAACTGGAGTGGCTCGGATACATCAGCTATTCCGGGTCCACATCCTACAATCCCTCTTTGAAATCCAGAATATCTATTACACGAGACACCAGCAAGAATCAATTCTTTCTGCAGTTGAATTCAGTGACCACCGAAGACACCGCCACTTACTACTGCGCGAAATCACAGCTGGGGAGATGGGCCATGGATTACTGGGGGCAGGGGACTAGCGTTACTGTTTCTTCAACAACTACGCCGGCGCCGAGACCACCTACACCTGCACCAACTATTGCCTCTCAGCCACTGAGTCTGCGCCCCGAGGCATGTCGACCTGCCGCTGGCGGGGCTGTGCACACCAGGGGCCTAGACTTCGCCTGCGATATCTATATTTGGGCTCCACTGGCAGGAACCTGTGGCGTGCTGCTGCTGTCTCTGGTCATCACACTGTACTGCAAAAGAGGCAGGAAGAAACTGCTGTATATTTTCAAGCAGCCCTTTATGAGACCTGTGCAGACAACTCAGGAGGAAGACGGGTGCAGCTGTAGGTTCCCTGAGGAAGAGGAAGGAGGCTGTGAGCTGCGCGTGAAATTTTCTCGGAGTGCAGATGCCCCAGCTTACCAGCAGGGCCAGAACCAGCTGTATAACGAGCTGAATCTGGGGCGGAGAGAGGAATACGACGTGCTGGATAAGAGGCGCGGGCGAGATCCAGAAATGGGAGGAAAACCCCAGCGACGGAAGAACCCTCAGGAGGGACTGTACAATGAACTGCAGAAGGACAAAATGGCAGAGGCCTATTCCGAAATCGGGATGAAAGGAGAAAGAAGGCGCGGCAAGGGGCATGATGGCCTGTATCAGGGACTGTCAACCGCAACAAAAGATACTTATGATGCTCTGCACATGCAGGCTCTGCCCCCGCGGTAA

SEQ ID NO: 54 - protein, 107 aa, synthetic construct
EIVLTQSPAILSLSPGERVTFSCRASQSIGTSIHWYQQKTNDSPRLLIKYASESISGIPSRFSGSGSGTDFTLNISSLESEDIADYYCQQSISWPLTFGPGTKLEIK

SEQ ID NO: 55 - protein, 120 aa, synthetic construct
EVQLLEQSGPGLVKPSQSLSLTCSVTGYSITSDYAWNWIRQFPGNKLEWIGYISYSGSTSYNPSLKSRVTITRDTSQNQYYLQLNSVTTEDTATYYCAKSQLGRWAMDYWGQGTTVTVSS

SEQ ID NO: 56 - protein, 107 aa, synthetic construct
EIVLTQSPAILSVSPGERVSFSCRASQNIGTSIHWYQQKTNGSPSLLIKYASESMSGIPSRFSGSGSGTDFTLTINSLQPEDIADYYCQQSNRWPYTFGGGTKLELK

SEQ ID NO: 57 - protein, 119 aa, synthetic construct
QLVQSGPELKKPGETVKISCKASGYSFTHYGVNWVRQAPGQGLEWMGWINTNTGKPTYAEDFKGRFAFSLDTSARTAYLQISSLKNEDTATYYCARWSTTVVAPYFDVWGAGTSVTVSS

SEQ ID NO: 58 - protein, 106 aa, synthetic construct
EIVLTQSPAILSASPGDRVTLSCSARSSVSYMNWYQQKSGSSPRIWIYGISNLASGIPARFSGSGSGTSFTFTINSMEAEDVAYYYCQLRSSYSRTFGGGTKVEIK

SEQ ID NO: 59 - protein, 121 aa, synthetic construct
QVQLQQSGAELVKPGTSVKISCKASGYTFTNYWLGWVKQRPGHGLEWIGDFYPGSIYTNYNENFQGKATLTADTSSSTAYMQLNSLTSEDTAVYFCAREGDYYGSGHFDYWGQGTTVTVSS

SEQ ID NO: 60 - protein, 268 aa, synthetic construct
MALPVTGLLLSLGLLLHAARPEIVLTQSPAILSLSPGERVTFSCRASQSIGTSIHWYQQKTNDSPRLLIKYASESISGIPSRFSGSGSGTDFTLNISSLESEDIADYYCQQSISWPLTFGPGTKLEIKGGGGSGGGGSGGGGSGGGGSEVQLLEQSGPGLVKPSQSLSLTCSVTGYSITSDYAWNWIRQFPGNKLEWIGYISYSGSTSYNPSLKSRVTITRDTSQNQYYLQLNSVTTEDTATYYCAKSQLGRWAMDYWGQGTTVTVSS

SEQ ID NO: 61 - protein, 267 aa, synthetic construct
MALPVTGLLLSLGLLLHAARPEIVLTQSPAILSVSPGERVSFSCRASQNIGTSIHWYQQKTNGSPSLLIKYASESMSGIPSRFSGSGSGTDFTLTINSLQPEDIADYYCQQSNRWPYTFGGGTKLELKGGGGSGGGGSGGGGSGGGGSQLVQSGPELKKPGETVKISCKASGYSFTHYGVNWVRQAPGQGLEWMGWINTNTGKPTYAEDFKGRFAFSLDTSARTAYLQISSLKNEDTATYYCARWSTTVVAPYFDVWGAGTSVTVSS

SEQ ID NO: 62 - protein, 268 aa, synthetic construct
MALPVTGLLLSLGLLLHAARPEIVLTQSPAILSASPGDRVTLSCSARSSVSYMNWYQQKSGSSPRIWIYGISNLASGIPARFSGSGSGTSFTFTINSMEAEDVAYYYCQLRSSYSRTFGGGTKVEIKGGGGSGGGGSGGGGSGGGGSQVQLQQSGAELVKPGTSVKISCKASGYTFTNYWLGWVKQRPGHGLEWIGDFYPGSIYTNYNENFQGKATLTADTSSSTAYMQLNSLTSEDTAVYFCAREGDYYGSGHFDYWGQGTTVTVSS

SEQ ID NO: 63 - protein, 294 aa, synthetic construct
MALPVTGLLLSLGLLLHAARPEILLTQSPAIIAASPGEKVTITCSARSSVSYMNWYQQKSGSSPKIWIYGISNLASGVPARFSGSGSGTSFSFTINSMEAEDVAYYYCQLRSSYSRTFGGGTKLEIKGGGGSGGGGSGGGGSGGGGSQVQLQQSGAELVRPGTSVKISCKASGYTFTNYWLGWVKQRPGHGLEWIGDFYPGSIYTNYNENFQGKATLTADTSSSTAYMQLSSLTSEDSAVYFCAREGDYYGSGHFDYWGQGTTLTVSSGGGGSGGGGSGGGGSGGGGSAEKDEL

SEQ ID NO: 64 - protein, 885 aa, synthetic construct
ATGGCTCTGCCTGTAACCGGACTCTTACTCTCTTTGGGGCTACTCCTTCACGCAGCCAGGCCTGAGATTCTGTTAACTCAGTCACCCGCTATTATTGCCGCATCTCCAGGCGAAAAGGTGACAATCACCTGCTCAGCCCGCAGCTCCGTATCTTACATGAACTGGTATCAGCAGAAATCAGGTTCATCCCCTAAGATATGGATCTATGGAATATCTAACTTGGCTTCAGGCGTGCCTGCAAGGTTCTCTGGGTCCGGTAGTGGCACTTCCTTTAGTTTCACAATCAATTCCATGGAAGCCGAGGATGTCGCATACTATTACTGTCAACTCAGAAGTTCCTACTCCCGTACATTCGGCGGCGGCACAAAACTTGAGATCAAGGGTGGGGGGGGTAGCGGAGGAGGCGGATCAGGAGGGGGCGGCAGTGGAGGCGGGGGCTCCCAGGTGCAGCTCCAGCAGTCCGGTGCCGAGCTGGTTCGGCCCGGCACATCCGTGAAGATCTCCTGCAAGGCTTCGGGCTATACTTTCACCAACTATTGGCTGGGATGGGTGAAACAAAGGCCCGGTCACGGGTTGGAGTGGATCGGGGATTTCTACCCTGGATCAATTTATACCAATTATAACGAGAATTTTCAAGGGAAAGCTACACTGACCGCCGACACTAGCAGCAGCACCGCCTACATGCAGCTCAGCTCTCTTACGAGCGAGGACTCGGCCGTCTACTTTTGTGCACGAGAAGGGGACTACTACGGCAGTGGTCATTTTGATTACTGGGGGCAGGGTACCACCCTCACGGTCAGCTCTGGCGGTGGCGGATCAGGTGGGGGCGGGTCTGGGGGCGGTGGCTCGGGCGGCGGGGGAAGTGCCGAGAAAGACGAACTCTAA

SEQ ID NO: 65 - protein, 492 aa, synthetic construct
MALPVTGLLLSLGLLLHAARPEIVLTQSPAILSLSPGERVTFSCRASQSIGTSIHWYQQKTNDSPRLLIKYASESISGIPSRFSGSGSGTDFTLNISSLESEDIADYYCQQSISWPLTFGPGTKLEIKGGGGSGGGGSGGGGSGGGGSEVQLLEQSGPGLVKPSQSLSLTCSVTGYSITSDYAWNWIRQFPGNKLEWIGYISYSGSTSYNPSLKSRVTITRDTSQNQYYLQLNSVTTEDTATYYCAKSQLGRWAMDYWGQGTTVTVSSTTTPAPRPPTPAPTIASQPLSLRPEACRPAAGGAVHTRGLDFACDIYIWAPLAGTCGVLLLSLVITLYCKRGRKKLLYIFKQPFMRPVQTTQEEDGCSCRFPEEEEGGCELRVKFSRSADAPAYQQGQNQLYNELNLGRREEYDVLDKRRGRDPEMGGKPQRRKNPQEGLYNELQKDKMAEAYSEIGMKGERRRGKGHDGLYQGLSTATKDTYDALHMQALPPR

SEQ ID NO: 66 - protein, 491 aa, synthetic construct
MALPVTGLLLSLGLLLHAARPEIVLTQSPAILSVSPGERVSFSCRASQNIGTSIHWYQQKTNGSPSLLIKYASESMSGIPSRFSGSGSGTDFTLTINSLQPEDIADYYCQQSNRWPYTFGGGTKLELKGGGGSGGGGSGGGGSGGGGSQLVQSGPELKKPGETVKISCKASGYSFTHYGVNWVRQAPGQGLEWMGWINTNTGKPTYAEDFKGRFAFSLDTSARTAYLQISSLKNEDTATYYCARWSTTVVAPYFDVWGAGTSVTVSSTTTPAPRPPTPAPTIASQPLSLRPEACRPAAGGAVHTRGLDFACDIYIWAPLAGTCGVLLLSLVITLYCKRGRKKLLYIFKQPFMRPVQTTQEEDGCSCRFPEEEEGGCELRVKFSRSADAPAYQQGQNQLYNELNLGRREEYDVLDKRRGRDPEMGGKPQRRKNPQEGLYNELQKDKMAEAYSEIGMKGERRRGKGHDGLYQGLSTATKDTYDALHMQALPPR

SEQ ID NO: 67 - protein, 294 aa, synthetic construct
MALPVTGLLLSLGLLLHAARPEIVLTQSPAILSLSPGERVTFSCRASQSIGTSIHWYQQKTNDSPRLLIKYASESISGIPSRFSGSGSGTDFTLNISSLESEDIADYYCQQSISWPLTFGPGTKLEIKGGGGSGGGGSGGGGSGGGGSEVQLLEQSGPGLVKPSQSLSLTCSVTGYSITSDYAWNWIRQFPGNKLEWIGYISYSGSTSYNPSLKSRVTITRDTSQNQYYLQLNSVTTEDTATYYCAKSQLGRWAMDYWGQGTTVTVSSGGGGSGGGGSGGGGSGGGGSAEKDEL

SEQ ID NO: 68 - protein, 293 aa, synthetic construct
MALPVTGLLLSLGLLLHAARPEIVLTQSPAILSVSPGERVSFSCRASQNIGTSIHWYQQKTNGSPSLLIKYASESMSGIPSRFSGSGSGTDFTLTINSLQPEDIADYYCQQSNRWPYTFGGGTKLELKGGGGSGGGGSGGGGSGGGGSQLVQSGPELKKPGETVKISCKASGYSFTHYGVNWVRQAPGQGLEWMGWINTNTGKPTYAEDFKGRFAFSLDTSARTAYLQISSLKNEDTATYYCARWSTTVVAPYFDVWGAGTSVTVSSGGGGSGGGGSGGGGSGGGGSAEKDEL

SEQ ID NO: 69 - protein, 294 aa, synthetic construct
MALPVTGLLLSLGLLLHAARPEIVLTQSPAILSASPGDRVTLSCSARSSVSYMNWYQQKSGSSPRIWIYGISNLASGIPARFSGSGSGTSFTFTINSMEAEDVAYYYCQLRSSYSRTFGGGTKVEIKGGGGSGGGGSGGGGSGGGGSQVQLQQSGAELVKPGTSVKISCKASGYTFTNYWLGWVKQRPGHGLEWIGDFYPGSIYTNYNENFQGKATLTADTSSSTAYMQLNSLTSEDTAVYFCAREGDYYGSGHFDYWGQGTTVTVSSGGGGSGGGGSGGGGSGGGGSAEKDEL

SEQ ID NO: 70 - protein, 492 aa, synthetic construct
MALPVTGLLLSLGLLLHAARPEIVLTQSPAILSASPGDRVTLSCSARSSVSYMNWYQQKSGSSPRIWIYGISNLASGIPARFSGSGSGTSFTFTINSMEAEDVAYYYCQLRSSYSRTFGGGTKVEIKGGGGSGGGGSGGGGSGGGGSQVQLQQSGAELVKPGTSVKISCKASGYTFTNYWLGWVKQRPGHGLEWIGDFYPGSIYTNYNENFQGKATLTADTSSSTAYMQLNSLTSEDTAVYFCAREGDYYGSGHFDYWGQGTTVTVSSTTTPAPRPPTPAPTIASQPLSLRPEACRPAAGGAVHTRGLDFACDIYIWAPLAGTCGVLLLSLVITLYCKRGRKKLLYIFKQPFMRPVQTTQEEDGCSCRFPEEEEGGCELRVKFSRSADAPAYQQGQNQLYNELNLGRREEYDVLDKRRGRDPEMGGKPQRRKNPQEGLYNELQKDKMAEAYSEIGMKGERRRGKGHDGLYQGLSTATKDTYDALHMQALPPR

SEQ ID NO: 71 - skipped

SEQ ID NO: 72 - DNA, 2424 bp, synthetic construct
  source 1..2424: mol_type = other DNA
atggctctgcctgtaaccggactcttactctctttggggctactccttcacgcagccaggcctgagatcgttcttacacagtcgccagccatcctgtctgtgtcccctggagagcgcgtctcatttagttgccgtgcttctcagaacatcggcaccagcatacattggtatcagcagaaaaccaacggctcccccagtttactgattaaatatgcttccgagtcaatgtctggtataccttccaggttctcaggttcaggaagcggcacagattttactcttacaatcaactctttgcagccagaagacattgcagactactactgtcaacagtctaatagatggccctatacgttcggtggaggcactaagttggagctcaaggggggcggaggtagtggaggcggcggcagcggaggcggggggtcggggggaggaggtagccaactagtgcaatccgggccagaactcaagaagccgggcgaaaccgtgaagatttcctgtaaagccagtggatacagcttcactcactacggcgtcaattgggtgcggcaggcccctgggcaggggctggagtggatggggtggattaataccaatacaggcaaacccacctatgctgaagactttaaagggaggttcgcattttccctggacacttctgcccgaaccgcctacctccagatcagcagcctgaagaacgaggatactgccacatactattgcgcgagatggagcacaaccgtagtcgcaccctacttcgatgtgtggggtgctggcacctcagtgacggttagttccacaactacgccggcgccgagaccacctacacctgcaccaactattgcctctcagccactgagtctgcgccccgaggcatgtcgacctgccgctggcggggctgtgcacaccaggggcctagacttcgcctgcgatatctatatttgggctccactggcaggaacctgtggcgtgctgctgctgtctctggtcatcacactgtactgcaaaagaggcaggaagaaactgctgtatattttcaagcagccctttatgagacctgtgcagacaactcaggaggaagacgggtgcagctgtaggttccctgaggaagaggaaggaggctgtgagctgcgcgtgaaattttctcggagtgcagatgccccagcttaccagcagggccagaaccagctgtataacgagctgaatctggggcggagagaggaatacgacgtgctggataagaggcgcgggcgagatccagaaatgggaggaaaaccccagcgacggaagaaccctcaggagggactgtacaatgaactgcagaaggacaaaatggcagaggcctattccgaaatcgggatgaaaggagaaagaaggcgcggcaaggggcatgatggcctgtatcagggactgtcaaccgcaacaaaagatacttatgatgctctgcacatgcaggctctgcccccgcggtctagagagggacgtggaagtctgctaacatgcggtgacgtcgaggagaatcccggccctacgcgtatggctctgcctgtaaccggactcttactctctttggggctactccttcacgcagccaggcctgaaatagtactgacacagtccccagcgattctcagcctgagccctggcgagagagtgactttttcttgtcgcgcctctcaatcaatcggaacttcaatccactggtaccagcagaaaaccaatgattcccctaggttgttaataaagtatgcatccgagtctatctctggaatcccctcgaggttcagtgggagcggcagcggtaccgattttacgttgaacatttcttccctggagagtgaagacatagctgattactactgccagcagagtattagttggccccttaccttcggcccggggacgaagctggagatcaagggagggggaggttcaggcggaggtgggtcaggcggcgggggatccgggggtggcgggtctgaagttcagctgctggaacagtcgggccccggtcttgtcaagcctagccaaagtctctcactgacttgtagcgtgaccggttatagcatcacaagtgactatgcctggaattggatccgtcagttcccaggcaataaactggagtggattggatatattagctatagcggctcaacatcctacaacccatccttaaagtcccgggtgactattactagagacacttcacagaaccagtactacctacaactcaacagcgtgaccacagaggacaccgcaacatactactgcgccaaatctcaactcgggcgatgggctatggattattggggacagggcaccacagtcaccgtttcttccggcggtggcggatcaggtgggggcgggtctgggggcggtggctcgggcggcgggggaagtgccgagaaagacgaactctaa

SEQ ID NO: 73 - protein, 807 aa, synthetic construct
MALPVTGLLLSLGLLLHAARPEIVLTQSPAILSVSPGERVSFSCRASQNIGTSIHWYQQKTNGSPSLLIKYASESMSGIPSRFSGSGSGTDFTLTINSLQPEDIADYYCQQSNRWPYTFGGGTKLELKGGGGSGGGGSGGGGSGGGGSQLVQSGPELKKPGETVKISCKASGYSFTHYGVNWVRQAPGQGLEWMGWINTNTGKPTYAEDFKGRFAFSLDTSARTAYLQISSLKNEDTATYYCARWSTTVVAPYFDVWGAGTSVTVSSTTTPAPRPPTPAPTIASQPLSLRPEACRPAAGGAVHTRGLDFACDIYIWAPLAGTCGVLLLSLVITLYCKRGRKKLLYIFKQPFMRPVQTTQEEDGCSCRFPEEEEGGCELRVKFSRSADAPAYQQGQNQLYNELNLGRREEYDVLDKRRGRDPEMGGKPQRRKNPQEGLYNELQKDKMAEAYSEIGMKGERRRGKGHDGLYQGLSTATKDTYDALHMQALPPRSREGRGSLLTCGDVEENPGPTRMALPVTGLLLSLGLLLHAARPEIVLTQSPAILSLSPGERVTFSCRASQSIGTSIHWYQQKTNDSPRLLIKYASESISGIPSRFSGSGSGTDFTLNISSLESEDIADYYCQQSISWPLTFGPGTKLEIKGGGGSGGGGSGGGGSGGGGSEVQLLEQSGPGLVKPSQSLSLTCSVTGYSITSDYAWNWIRQFPGNKLEWIGYISYSGSTSYNPSLKSRVTITRDTSQNQYYLQLNSVTTEDTATYYCAKSQLGRWAMDYWGQGTTVTVSSGGGGSGGGGSGGGGSGGGGSAEKDEL

SEQ ID NO: 74 - DNA, 2421 bp, synthetic construct
  source 1..2421: mol_type = other DNA
atggctctgcctgtaaccggactcttactctctttggggctactccttcacgcagccaggcctgacattctgctgactcagtcaccagccatcctctcagtgtcacctggcgagcgtgtttcattcagctgtagggcttcgcaaaatatcgggaccagcatccactggttccagcagagatctaacggctcgccaagcttactcatcaaatatgcgagtgagtccatgtccggcatcccttcacgcttttccggctctggttctggaactgattttacccttagcataaatagtgtggagcctgaagatatagccgactactactgccaacaatccaaccggtggccctacacatttggcggtggcaccaaacttgagattaagggtggggggggtagcggaggaggcggatcaggagggggcggcagtggaggcgggggctcccagctagtgcagtctggacccgaagtgaaaaagcctggagagacagttaagatttcctgcaaagcaagtggatatagcttcacacactacggtgtaaattgggtgaagcaggcaccaggcaaagggcttaagtggatggggtggatcaacacaaatacgggcaagcccacttatgccgaagactttaaggggagattcgccttctctctggaaacgagtgcacgaacagcttacctccagattaacaatctgaaaaacgaggatactgctacatatttctgtgctaggtggtcaaccaccgtcgtggccccctactttgacgtctggggtgcggggactaccgtaaccgtctcctccacaactacgccggcgccgagaccacctacacctgcaccaactattgcctctcagccactgagtctgcgccccgaggcatgtcgacctgccgctggcggggctgtgcacaccaggggcctagacttcgcctgcgatatctatatttgggctccactggcaggaacctgtggcgtgctgctgctgtctctggtcatcacactgtactgcaaaagaggcaggaagaaactgctgtatattttcaagcagccctttatgagacctgtgcagacaactcaggaggaagacgggtgcagctgtaggttccctgaggaagaggaaggaggctgtgagctgcgcgtgaaattttctcggagtgcagatgccccagcttaccagcagggccagaaccagctgtataacgagctgaatctggggcggagagaggaatacgacgtgctggataagaggcgcgggcgagatccagaaatgggaggaaaaccccagcgacggaagaaccctcaggagggactgtacaatgaactgcagaaggacaaaatggcagaggcctattccgaaatcgggatgaaaggagaaagaaggcgcggcaaggggcatgatggcctgtatcagggactgtcaaccgcaacaaaagatacttatgatgctctgcacatgcaggctctgcccccgcggtctagagagggacgtggaagtctgctaacatgcggtgacgtcgaggagaatcccggccctacgcgtatggctctgcctgtaaccggactcttactctctttggggctactccttcacgcagccaggcctgacattctgcttacacagagtcccgccatcctgagcgtctctccaggcgagcgggtctccttcagttgtcgcgctagtcagagcattggaacctccatccattggtatcagcagagaacgaatgatagcccccggctgctgataaagtatgcatccgagtccatatcaggcatcccttctaggttttcaggaagcggatctggcactgactttacgttgaacatcaacagcgtggaatccgaggacatcgctgattattattgccaacagtctatctcctggccgcttacattcggcccaggaacaaagttagagctgaagggtggggggggtagcggaggaggcggatcaggagggggcggcagtggaggcgggggctccgatgtgcagctgcaagaaagtggcccaggtcttgtgaagcctagtcagagcctgagcctaacctgtacagtgaccggttacagcattacttcggattacgcatggaactggattcgtcaattccccggtaacaaactggagtggctcggatacatcagctattccgggtccacatcctacaatccctctttgaaatccagaatatctattacacgagacaccagcaagaatcaattctttctgcagttgaattcagtgaccaccgaagacaccgccacttactactgcgcgaaatcacagctggggagatgggccatggattactgggggcaggggactagcgttactgtttcttcaggcggtggcggatcaggtgggggcgggtctgggggcggtggctcgggcggcgggggaagtgccgagaaagacgaactctaa

SEQ ID NO: 75 - protein, 806 aa, synthetic construct
MALPVTGLLLSLGLLLHAARPDILLTQSPAILSVSPGERVSFSCRASQNIGTSIHWFQQRSNGSPSLLIKYASESMSGIPSRFSGSGSGTDFTLSINSVEPEDIADYYCQQSNRWPYTFGGGTKLEIKGGGGSGGGGSGGGGSGGGGSQLVQSGPEVKKPGETVKISCKASGYSFTHYGVNWVKQAPGKGLKWMGWINTNTGKPTYAEDFKGRFAFSLETSARTAYLQINNLKNEDTATYFCARWSTTVVAPYFDVWGAGTTVTVSSTTTPAPRPPTPAPTIASQPLSLRPEACRPAAGGAVHTRGLDFACDIYIWAPLAGTCGVLLLSLVITLYCKRGRKKLLYIFKQPFMRPVQTTQEEDGCSCRFPEEEEGGCELRVKFSRSADAPAYQQGQNQLYNELNLGRREEYDVLDKRRGRDPEMGGKPQRRKNPQEGLYNELQKDKMAEAYSEIGMKGERRRGKGHDGLYQGLSTATKDTYDALHMQALPPRSREGRGSLLTCGDVEENPGPTRMALPVTGLLLSLGLLLHAARPDILLTQSPAILSVSPGERVSFSCRASQSIGTSIHWYQQRTNDSPRLLIKYASESISGIPSRFSGSGSGTDFTLNINSVESEDIADYYCQQSISWPLTFGPGTKLELKGGGGSGGGGSGGGGSGGGGSDVQLQESGPGLVKPSQSLSLTCTVTGYSITSDYAWNWIRQFPGNKLEWLGYISYSGSTSYNPSLKSRISITRDTSKNQFFLQLNSVTTEDTATYYCAKSQLGRWAMDYWGQGTSVTVSSGGGGSGGGGSGGGGSGGGGSAEKDEL

SEQ ID NO: 76 - DNA, 2427 bp, synthetic construct
  source 1..2427: mol_type = other DNA
atggctctgcctgtaaccggactcttactctctttggggctactccttcacgcagccaggcctgagatcgtgctgacccagagcccagctatcctgagtgcctctccaggggatagagtaactctttcgtgttccgcccgtagtagtgtctcttacatgaactggtaccagcagaaatcaggcagcagcccccgcatttggatttacggtatcagcaacctcgccagcggtattcctgccagattcagcggatccgggtcagggactagcttcacattcacaatcaatagcatggaggctgaagacgtggcctattattattgtcagttaaggtcctcctactcgaggacatttgggggaggcaccaaggtggagattaagggcggcgggggctcagggggcggcggttcaggcgggggcggatctggaggaggaggcagtcaggtgcagctgcagcaatccggcgcagaactcgtgaagcctggcacatctgtcaagataagttgcaaggcttccggatatacttttaccaattattggttgggttgggtgaaacaacggccgggacatggtctagagtggatcggggatttttaccccggtagtatatatactaactacaatgaaaactttcagggaaaagccacccttaccgctgacacttcctcctctacagcatacatgcagctgaattcactgacgtctgaagacaccgcagtctacttctgcgcgcgagagggggattactatgggtctggccacttcgactactggggacaaggcacaaccgttacggttagctcaacaactacgccggcgccgagaccacctacacctgcaccaactattgcctctcagccactgagtctgcgccccgaggcatgtcgacctgccgctggcggggctgtgcacaccaggggcctagacttcgcctgcgatatctatatttgggctccactggcaggaacctgtggcgtgctgctgctgtctctggtcatcacactgtactgcaaaagaggcaggaagaaactgctgtatattttcaagcagccctttatgagacctgtgcagacaactcaggaggaagacgggtgcagctgtaggttccctgaggaagaggaaggaggctgtgagctgcgcgtgaaattttctcggagtgcagatgccccagcttaccagcagggccagaaccagctgtataacgagctgaatctggggcggagagaggaatacgacgtgctggataagaggcgcgggcgagatccagaaatgggaggaaaaccccagcgacggaagaaccctcaggagggactgtacaatgaactgcagaaggacaaaatggcagaggcctattccgaaatcgggatgaaaggagaaagaaggcgcggcaaggggcatgatggcctgtatcagggactgtcaaccgcaacaaaagatacttatgatgctctgcacatgcaggctctgcccccgcggtctagagagggacgtggaagtctgctaacatgcggtgacgtcgaggagaatcccggccctacgcgtatggctctgcctgtaaccggactcttactctctttggggctactccttcacgcagccaggcctgaaatagtactgacacagtccccagcgattctcagcctgagccctggcgagagagtgactttttcttgtcgcgcctctcaatcaatcggaacttcaatccactggtaccagcagaaaaccaatgattcccctaggttgttaataaagtatgcatccgagtctatctctggaatcccctcgaggttcagtgggagcggcagcggtaccgattttacgttgaacatttcttccctggagagtgaagacatagctgattactactgccagcagagtattagttggccccttaccttcggcccggggacgaagctggagatcaagggagggggaggttcaggcggaggtgggtcaggcggcgggggatccgggggtggcgggtctgaagttcagctgctggaacagtcgggccccggtcttgtcaagcctagccaaagtctctcactgacttgtagcgtgaccggttatagcatcacaagtgactatgcctggaattggatccgtcagttcccaggcaataaactggagtggattggatatattagctatagcggctcaacatcctacaacccatccttaaagtcccgggtgactattactagagacacttcacagaaccagtactacctacaactcaacagcgtgaccacagaggacaccgcaacatactactgcgccaaatctcaactcgggcgatgggctatggattattggggacagggcaccacagtcaccgtttcttccggcggtggcggatcaggtgggggcgggtctgggggcggtggctcgggcggcgggggaagtgccgagaaagacgaactctaa

SEQ ID NO: 77 - protein, 808 aa, synthetic construct
MALPVTGLLLSLGLLLHAARPEIVLTQSPAILSASPGDRVTLSCSARSSVSYMNWYQQKSGSSPRIWIYGISNLASGIPARFSGSGSGTSFTFTINSMEAEDVAYYYCQLRSSYSRTFGGGTKVEIKGGGGSGGGGSGGGGSGGGGSQVQLQQSGAELVKPGTSVKISCKASGYTFTNYWLGWVKQRPGHGLEWIGDFYPGSIYTNYNENFQGKATLTADTSSSTAYMQLNSLTSEDTAVYFCAREGDYYGSGHFDYWGQGTTVTVSSTTTPAPRPPTPAPTIASQPLSLRPEACRPAAGGAVHTRGLDFACDIYIWAPLAGTCGVLLLSLVITLYCKRGRKKLLYIFKQPFMRPVQTTQEEDGCSCRFPEEEEGGCELRVKFSRSADAPAYQQGQNQLYNELNLGRREEYDVLDKRRGRDPEMGGKPQRRKNPQEGLYNELQKDKMAEAYSEIGMKGERRRGKGHDGLYQGLSTATKDTYDALHMQALPPRSREGRGSLLTCGDVEENPGPTRMALPVTGLLLSLGLLLHAARPEIVLTQSPAILSLSPGERVTFSCRASQSIGTSIHWYQQKTNDSPRLLIKYASESISGIPSRFSGSGSGTDFTLNISSLESEDIADYYCQQSISWPLTFGPGTKLEIKGGGGSGGGGSGGGGSGGGGSEVQLLEQSGPGLVKPSQSLSLTCSVTGYSITSDYAWNWIRQFPGNKLEWIGYISYSGSTSYNPSLKSRVTITRDTSQNQYYLQLNSVTTEDTATYYCAKSQLGRWAMDYWGQGTTVTVSSGGGGSGGGGSGGGGSGGGGSAEKDEL